European Patent Specification EP 4 244 238 B1, published January 29, 2025. Title: Binding proteins for Complement Factor H (CFH). Applicant: Navigo Proteins GmbH. The sequence listing filed with the application follows.

SEQUENCE LISTING (28 sequences)

SEQ ID NO: 1 - protein, 58 aa, Artificial Sequence
  CFH binding protein 209202
NAADLDEAQISAIFEIMDLPNLTWQQQEWFIDSLSDDPSVSKEVLGEAQKLNDSQAPK

SEQ ID NO: 2 - protein, 58 aa, Artificial Sequence
  CFH binding protein 209264
IAAKFDRIQSIADEVILILPNLTEEQRNAFRQSLSDDPSVSEEVLYEALYLNYSQAPK

SEQ ID NO: 3 - protein, 58 aa, Artificial Sequence
  CFH binding protein 209274
IAARFDKAQRAAELEIKALPNLTYEQRKAFRVSLYDDPSVSLEVLGEAQKLNDSQAPK

SEQ ID NO: 4 - protein, 58 aa, Artificial Sequence
  CFH binding protein 209275
IAARFDHAQWAAELEIKELPNLTYEQRKAFRISLYDDPSVSLEVLGEAQKLNDSQAPK

SEQ ID NO: 5 - protein, 58 aa, Artificial Sequence
  CFH binding protein 209447
NAAEADDAQVSAAMEIIMLPNLTLEQAHSFIESLYRDPSVSKEVLGEAQKLNDSQAPK

SEQ ID NO: 6 - protein, 58 aa, Artificial Sequence
  CFH binding protein 209466
NAADKDFAQESAEYEILMLPNLTLDQAYSFILSLKSDPSVSKEVLGEAQKLNDSQAPK

SEQ ID NO: 7 - protein, 116 aa, Artificial Sequence
  CFH binding protein 208851
IAAKFDEAQWAAFYEIVHLPNLTEEQREAFIQSLWDDPGVSLEVLGEAQKLNDSQAPKIAAKFDEAQQAAFYEILHLPNLTEAQRNHFIQRLRDDPSVSLVVLGQAQKLNDSQAPK

SEQ ID NO: 8 - protein, 116 aa, Artificial Sequence
  CFH binding protein 208854
IAAKFDEAQQKAFYWILHLRNLTEEQRNAFIQSLRDDPSVSTEVLGEALKLNQSQAPKIAAKFDEAQWAAFYEIVHLPNLTEEQREAFIQSLWDDPSVSLEVLGEAQKLNDSQAPK

SEQ ID NO: 9 - protein, 116 aa, Artificial Sequence
  CFH binding protein 209354
IAAKFDEAQWAAFYEIVHLPNLTEEQREAFIQSLWDDPSVSLEVLGEAQKLNDSQAPKIAAKFDEAQQAAFYEILHLPNLTEHQRNHFIQKLRDDPSVSLQVLGHAQRLNDSQAPK

SEQ ID NO: 10 - protein, 116 aa, Artificial Sequence
  CFH binding protein 209372
IAAKFDEAQWAAFYEIVHLPNLTEEQREAFIQSLWDDPSVSLEVLGEAQKLNDSQAPKIAAKFDEAQQAAFYEILHLPNLTEQQRNYFIQRLRDDPSVSLAVLGHAQKLNDSQAPK

SEQ ID NO: 11 - protein, 116 aa, Artificial Sequence
  CFH binding protein 209429
IAAKFDEAQQRAFYWILHLRNLTEEQRNAFIQSLRDDPSVSKEVLGEAYKLNKSQAPKIAAKFDEAQTAAFWEIWHLPNLTEEQRVAFIHSLQDDPSVSLEVLGEAQKLNDSQAPK

SEQ ID NO: 12 - protein, 116 aa, Artificial Sequence
  CFH binding protein 209434
IAAKFDEAQQRAFYWILHLRNLTEEQRNAFIQSLRDDPSVSKEVLGEAYKLNVSQAPKIAAKFDEAQVAAFWEIWHLPNLTEEQRVAFIHSLQDDQSVSLEVLGEAQKLNDSQAPK

SEQ ID NO: 13 - protein, 116 aa, Artificial Sequence
  CFH binding protein 209621
IAAKFDEAQTAAFWEIEHLPNLTEEQRWAFIWSLADDPSVSLEVLGEAQKLNDSQAPKIAAKFDEAQQAAFYEILHLPNLTEWQRNYFIQKLRDDPSVSLWVLGQAQILNDSQAPK

SEQ ID NO: 14 - protein, 116 aa, Artificial Sequence
  CFH binding protien 209826
IAAKFDEAQEAAFWEIQHLPNLTEEQRWAFIWSLADDPSVSLEVLGEAQKLNDSQAPKIAAKFDEAQQAAFYEILHLPNLTEYQRNLFIQRLRDDPSVSLWVLGQAQILNDSQAPK

SEQ ID NO: 15 - protein, 116 aa, Artificial Sequence
  CFH binding protein 209827
IAAKFDEAQEAAFWEIQHLPNLTEEQRWAFIWSLADDPSVSLEVLGEAQKLNDSQAPKIAAKFDEAQQAAFYEILHLPNLTEWQRNYFIQKLRDDPSVSLWVLGQAQILNDSQAPK

SEQ ID NO: 16 - protein, 116 aa, Artificial Sequence
  CFH binding protein 209831
IAAKFDEAQWAAFYEIVHLPNLTEEQREAFIQSLWDDPSVSLEVLGEAQKLNDSQAPKIAAKFDEAQQAAFYEILHLPNLTERQRNWFIQRLRDDPSVSLWVLGRAQRLNDSQAPK

SEQ ID NO: 17 - protein, 116 aa, Artificial Sequence
  CFH binding protein 209833
IAAKFDEAQEAAFWEIQHLPNLTEEQRWAFIWSLADDPSVSLEVLGEAQKLNDSQAPKIAAKFDEAQQAAFYEILHLPNLTEHQRNLFIQRLRDDPSVSLWVLGQAQILNDSQAPK

SEQ ID NO: 18 - protein, 116 aa, Artificial Sequence
  CFH binding protein 209835
IAAKFDEAQWAAFYEIVHLPNLTEEQREAFIQSLWDDPSVSLEVLGEAQKLNDSQAPKIAAKFDEAQQAAFYEILHLPNLTERQRNWFIQQLRDDPSVSLTVLGRAQRLNDSQAPK

SEQ ID NO: 19 - protein, 116 aa, Artificial Sequence
  CFH binding protien 209860
IAAKFDEAQWAAFEEIAHLPNLTEEQREAFIQSLWDDPSVSLEVLGEAQKLNDSQAPKIAAKFDEAQQAAFYEILHLPNLTERQRNWFIQRLRDDPSVSLWVLGRAQRLNDSQAPK

SEQ ID NO: 20 - protein, 116 aa, Artificial Sequence
  CFH binding protein 209864
IAAKFDEAQQAAFYEILHLPNLTELQRNHFIQTLRDDPSVSLWVLGLAQLLNDSQAPKIAAKFDEAQQHAFYTILHLENLTEEQRNAFIQSLRDDPSVSLEVLGEAIKLNISQAPK

SEQ ID NO: 21 - protein, 116 aa, Artificial Sequence
  CFH binding protein 209920
IAAKFDEAQQEAFYWILHLENLTEEQRNAFIQSLRDDPSVSEEVLGEALKLNVSQAPKIAAKFDEAQYAAFWEIQHLPNLTEEQRHAFIWSLLDDPSVSLEVLGEAQKLNDSQAPK

SEQ ID NO: 22 - protein, 117 aa, Artificial Sequence
  CFH binding protein 209921
IAAKFDEAQQEWAFYHILHLYNLTEEQRNAFIQSLRDDPSVSQEVLGEAWKLNQSQAPKIAAKFDEAQYAAFWEIWHLPNLTEEQRWAFILSLHDDPSVSLEVLGEAQKLNDSQAPK

SEQ ID NO: 23 - protein, 114 aa, Artificial Sequence
  CFH binding protein 213108 (SEQ13/209621variant del2N)
AKFDEAQTAAFWEIEHLPNLTEEQRWAFIWSLADDPSVSLEVLGEAQKLNDSQAPKIAAKFDEAQQAAFYEILHLPNLTEWQRNYFIQKLRDDPSVSLWVLGQAQILNDSQAPK

SEQ ID NO: 24 - protein, 250 aa, Artificial Sequence
  CFH binding protein 213109 (209621 delN dimer)
AKFDEAQTAAFWEIEHLPNLTEEQRWAFIWSLADDPSVSLEVLGEAQKLNDSQAPKIAAKFDEAQQAAFYEILHLPNLTEWQRNYFIQKLRDDPSVSLWVLGQAQILNDSQAPKQAPKVDAKFDQAPKVDAKFDIAAKFDEAQTAAFWEIEHLPNLTEEQRWAFIWSLADDPSVSLEVLGEAQKLNDSQAPKIAAKFDEAQQAAFYEILHLPNLTEWQRNYFIQKLRDDPSVSLWVLGQAQILNDSQAPK

SEQ ID NO: 25 - protein, 288 aa, Artificial Sequence
  CFH binding protien 213110 (209621 delN fusion with PAdelFc trimer)
AKFDEAQTAAFWEIEHLPNLTEEQRWAFIWSLADDPSVSLEVLGEAQKLNDSQAPKIAAKFDEAQQAAFYEILHLPNLTEWQRNYFIQKLRDDPSVSLWVLGQAQILNDSQAPKIAAQHDKIQQAADKEILHLPNLTEEQRNKFRQSLRDDPSVSAEILAEAKKLNDAQAPKIAAQHDKIQQAADKEILHLPNLTEEQRNKFRQSLRDDPSVSAEILAEAKKLNDAQAPKIAAQHDKIQQAADKEILHLPNLTEEQRNKFRQSLRDDPSVSAEILAEAKKLNDAQAPK

SEQ ID NO: 26 - protein, 58 aa, Artificial Sequence
  PAdelFc (non Ig binding protein)
IAAQHDKIQQAADKEILHLPNLTEEQRNKFRQSLRDDPSVSAEILAEAKKLNDAQAPK

SEQ ID NO: 27 - protein, 11 aa, Artificial Sequence
  coupling and Streptag
CSAWSHPQFEK

SEQ ID NO: 28 - protein, 10 aa, Artificial Sequence
  streptag
SAWSHPQFEK